European Patent Specification EP 3 347 371 B1, published May 10, 2023. Title: Treatment of retinitis pigmentosa. Applicant: Oxford University Innovation Limited. The sequence listing filed with the application follows.

SEQUENCE LISTING (14 sequences)

SEQ ID NO: 1 - protein, 1152 aa, Homo sapiens
MREPEELMPDSGAVFTFGKSKFAENNPGKFWFKNDVPVHLSCGDEHSAVVTGNNKLYMFGSNNWGQLGLGSKSAISKPTCVKALKPEKVKLAACGRNHTLVSTEGGNVYATGGNNEGQLGLGDTEERNTFHVISFFTSEHKIKQLSAGSNTSAALTEDGRLFMWGDNSEGQIGLKNVSNVCVPQQVTIGKPVSWISCGYYHSAFVTTDGELYVFGEPENGKLGLPNQLLGNHRTPQLVSEIPEKVIQVACGGEHTVVLTENAVYTFGLGQFGQLGLGTFLFETSEPKVIENIRDQTISYISCGENHTALITDIGLMYTFGDGRHGKLGLGLENFTNHFIPTLCSNFLRFIVKLVACGGCHMVVFAAPHRGVAKEIEFDEINDTCLSVATFLPYSSLTSGNVLQRTLSARMRRRERERSPDSFSMRRTLPPIEGTLGLSACFLPNSVFPRCSERNLQESVLSEQDLMQPEEPDYLLDEMTKEAEIDNSSTVESLGETTDILNMTHIMSLNSNEKSLKLSPVQKQKKQQTIGELTQDTALTENDDSDEYEEMSEMKEGKACKQHVSQGIFMTQPATTIEAFSDEEVEIPEEKEGAEDSKGNGIEEQEVEANEENVKVHGGRKEKTEILSDDLTDKAEVSEGKAKSVGEAEDGPEGRGDGTCEEGSSGAEHWQDEEREKGEKDKGRGEMERPGEGEKELAEKEEWKKRDGEEQEQKEREQGHQKERNQEMEEGGEEEHGEGEEEEGDREEEEEKEGEGKEEGEGEEVEGEREKEEGERKKEERAGKEEKGEEEGDQGEGEEEETEGRGEEKEEGGEVEGGEVEEGKGEREEEEEEGEGEEEEGEGEEEEGEGEEEEGEGKGEEEGEEGEGEEEGEEGEGEGEEEEGEGEGEEEGEGEGEEEEGEGEGEEEGEGEGEEEEGEGKGEEEGEEGEGEGEEEEGEGEGEDGEGEGEEEEGEWEGEEEEGEGEGEEEGEGEGEEGEGEGEEEEGEGEGEEEEGEEEGEEEGEGEEEGEGEGEEEEEGEVEGEVEGEEGEGEGEEEEGEEEGEEREKEGEGEENRRNREEEEEEEGKYQETGEEENERQDGEEYKKVSKIKGSVKYGKHKTYQKKSVTNTQGNGKEQRSKMPVQSKRLLKNGPSGSKKFWNNVLPHYLELK

SEQ ID NO: 2 - DNA, 3459 bp, Homo sapiens
atgagggagccggaagagctgatgcccgattcgggtgctgtgtttacatttgggaaaagtaaatttgctgaaaataatcccggtaaattctggtttaaaaatgatgtccctgtacatctttcatgtggagatgaacattctgctgttgttaccggaaataataaactttacatgtttggcagtaacaactggggtcagttaggattaggatcaaagtcagccatcagcaagccaacatgtgtcaaagctctaaaacctgaaaaagtgaaattagctgcctgtggaaggaaccacaccctggtgtcaacagaaggaggcaatgtatatgcaactggtggaaataatgaaggacagttggggcttggtgacaccgaagaaagaaacacttttcatgtaattagcttttttacatccgagcataagattaagcagctgtctgctggatctaatacttcagctgccctaactgaggatggaagactttttatgtggggtgacaattccgaagggcaaattggtttaaaaaatgtaagtaatgtctgtgtccctcagcaagtgaccattgggaaacctgtctcctggatctcttgtggatattaccattcagcttttgtaacaacagatggtgagctatatgtgtttggagaacctgagaatgggaagttaggtcttcccaatcagctcctgggcaatcacagaacaccccagctggtgtctgaaattccggagaaggtgatccaagtagcctgtggtggagagcatactgtggttctcacggagaatgctgtgtatacctttgggctgggacaatttggtcagctgggtcttggcacttttctttttgaaacttcagaacccaaagtcattgagaatattagggatcaaacaataagttatatttcttgtggagaaaatcacacagctttgataacagatatcggccttatgtatacttttggagatggtcgccacggaaaattaggacttggactggagaattttaccaatcacttcattcctactttgtgctctaattttttgaggtttatagttaaattggttgcttgtggtggatgtcacatggtagtttttgctgctcctcatcgtggtgtggcaaaagaaattgaattcgatgaaataaatgatacttgcttatctgtggcgacttttctgccgtatagcagtttaacctcaggaaatgtactgcagaggactctatcagcacgtatgcggcgaagagagagggagaggtctccagattctttttcaatgaggagaacactacctccaatagaagggactcttggcctttctgcttgttttctccccaattcagtctttccacgatgttctgagagaaacctccaagagagtgtcttatctgaacaggacctcatgcagccagaggaaccagattatttgctagatgaaatgaccaaagaagcagagatagataattcttcaactgtagaaagccttggagaaactactgatatcttaaacatgacacacatcatgagcctgaattccaatgaaaagtcattaaaattatcaccagttcagaaacaaaagaaacaacaaacaattggggaactgacgcaggatacagctcttactgaaaacgatgatagtgatgaatatgaagaaatgtcagaaatgaaagaagggaaagcatgtaaacaacatgtgtcacaagggattttcatgacgcagccagctacgactatcgaagcattttcagatgaggaagtagagatcccagaggagaaggaaggagcagaggattcaaaaggaaatggaatagaggagcaagaggtagaagcaaatgaggaaaatgtgaaggtgcatggaggaagaaaggagaaaacagagatcctatcagatgaccttacagacaaagcagaggtgagtgaaggcaaggcaaaatcagtgggagaagcagaggatgggcctgaaggtagaggggatggaacctgtgaggaaggtagttcaggagcagaacactggcaagatgaggagagggagaagggggagaaagacaagggtagaggagaaatggagaggccaggagagggagagaaggaactagcagagaaggaagaatggaagaagagggatggggaagagcaggagcaaaaggagagggagcagggccatcagaaggaaagaaaccaagagatggaggagggaggggaggaggagcatggagaaggagaagaagaggagggagacagagaagaggaagaagagaaggagggagaagggaaagaggaaggagaaggggaagaagtggagggagaacgtgaaaaggaggaaggagagaggaaaaaggaggaaagagcggggaaggaggagaaaggagaggaagaaggagaccaaggagagggggaagaggaggaaacagaggggagaggggaggaaaaagaggagggaggggaagtagagggaggggaagtagaggaggggaaaggagagagggaagaggaagaggaggagggtgagggggaagaggaggaaggggagggggaagaggaggaaggggagggggaagaggaggaaggagaagggaaaggggaggaagaaggggaagaaggagaaggggaggaagaaggggaggaaggagaaggggagggggaagaggaggaaggagaaggggagggagaagaggaaggagaaggggagggagaagaggaggaaggagaaggggagggagaagaggaaggagaaggggagggagaagaggaggaaggagaagggaaaggggaggaggaaggagaggaaggagaaggggagggggaagaggaggaaggagaaggggaaggggaggatggagaaggggagggggaagaggaggaaggagaatgggagggggaagaggaggaaggagaaggggagggggaagaggaaggagaaggggaaggggaggaaggagaaggggagggggaagaggaggaaggagaaggggagggggaagaggaggaaggggaagaagaaggggaggaagaaggagagggagaggaagaaggggagggagaaggggaggaagaagaggaaggggaagtggaaggggaggtggaaggggaggaaggagagggggaaggagaggaagaggaaggagaggaggaaggagaagaaagggaaaaggagggggaaggagaagaaaacaggaggaacagagaagaggaggaggaagaagaggggaagtatcaggagacaggcgaagaagagaatgaaaggcaggatggagaggagtacaaaaaagtgagcaaaataaaaggatctgtgaaatatggcaaacataaaacatatcaaaaaaagtcagttactaacacacagggaaatgggaaagagcagaggtccaaaatgccagtccagtcaaaacgacttttaaaaaacgggccatcaggttccaaaaagttctggaataatgtattaccacattacttggaattgaagtaa

SEQ ID NO: 3 - DNA, 3459 bp, Artificial Sequence
  codon-optimised sequence of RPGRORF15
atgagagagccagaggagctgatgccagacagtggagcagtgtttacattcggaaaatctaagttcgctgaaaataacccaggaaagttctggtttaaaaacgacgtgcccgtccacctgtcttgtggcgatgagcatagtgccgtggtcactgggaacaataagctgtacatgttcgggtccaacaactggggacagctggggctgggatccaaatctgctatctctaagccaacctgcgtgaaggcactgaaacccgagaaggtcaaactggccgcttgtggcagaaaccacactctggtgagcaccgagggcgggaatgtctatgccaccggaggcaacaatgagggacagctgggactgggggacactgaggaaaggaatacctttcacgtgatctccttctttacatctgagcataagatcaagcagctgagcgctggctccaacacatctgcagccctgactgaggacgggcgcctgttcatgtggggagataattcagagggccagattgggctgaaaaacgtgagcaatgtgtgcgtccctcagcaggtgaccatcggaaagccagtcagttggatttcatgtggctactatcatagcgccttcgtgaccacagatggcgagctgtacgtctttggggagcccgaaaacggaaaactgggcctgcctaaccagctgctgggcaatcaccggacaccccagctggtgtccgagatccctgaaaaagtgatccaggtcgcctgcgggggagagcatacagtggtcctgactgagaatgctgtgtataccttcggactgggccagtttggccagctggggctgggaaccttcctgtttgagacatccgaaccaaaagtgatcgagaacattcgcgaccagactatcagctacatttcctgcggagagaatcacaccgcactgatcacagacattggcctgatgtatacctttggcgatggacgacacgggaagctgggactgggactggagaacttcactaatcattttatccccaccctgtgttctaacttcctgcggttcatcgtgaaactggtcgcttgcggcgggtgtcacatggtggtcttcgctgcacctcataggggcgtggctaaggagatcgaatttgacgagattaacgatacatgcctgagcgtggcaactttcctgccatacagctccctgacttctggcaatgtgctgcagagaaccctgagtgcaaggatgcggagaagggagagggaacgctctcctgacagtttctcaatgcgacgaaccctgccacctatcgagggaacactgggactgagtgcctgcttcctgcctaactcagtgtttccacgatgtagcgagcggaatctgcaggagtctgtcctgagtgagcaggatctgatgcagccagaggaacccgactacctgctggatgagatgaccaaggaggccgaaatcgacaactctagtacagtggagtccctgggcgagactaccgatatcctgaatatgacacacattatgtcactgaacagcaatgagaagagtctgaaactgtcaccagtgcagaagcagaagaaacagcagactattggcgagctgactcaggacaccgccctgacagagaacgacgatagcgatgagtatgaggaaatgtccgagatgaaggaaggcaaagcttgtaagcagcatgtcagtcaggggatcttcatgacacagccagccacaactattgaggctttttcagacgaggaagtggagatccccgaggaaaaagagggcgcagaagattccaaggggaatggaattgaggaacaggaggtggaagccaacgaggaaaatgtgaaagtccacggaggcaggaaggagaaaacagaaatcctgtctgacgatctgactgacaaggccgaggtgtccgaaggcaaggcaaaatctgtcggagaggcagaagacggaccagagggacgaggggatggaacctgcgaggaaggctcaagcggggctgagcattggcaggacgaggaacgagagaagggcgaaaaggataaaggccgcggggagatggaacgacctggagagggcgaaaaagagctggcagagaaggaggaatggaagaaaagggacggcgaggaacaggagcagaaagaaagggagcagggccaccagaaggagcgcaaccaggagatggaagagggcggcgaggaagagcatggcgagggagaagaggaagagggcgatagagaagaggaagaggaaaaagaaggcgaagggaaggaggaaggagagggcgaggaagtggaaggcgagagggaaaaggaggaaggagaacggaagaaagaggaaagagccggcaaagaggaaaagggcgaggaagagggcgatcagggcgaaggcgaggaggaagagaccgagggccgcggggaagagaaagaggagggaggagaggtggagggcggagaggtcgaagagggaaagggcgagcgcgaagaggaagaggaagagggcgagggcgaggaagaagagggcgagggggaagaagaggagggagagggcgaagaggaagagggggagggaaagggcgaagaggaaggagaggaaggggagggagaggaagagggggaggagggcgagggggaaggcgaggaggaagaaggagagggggaaggcgaagaggaaggcgagggggaaggagaggaggaagaaggggaaggcgaaggcgaagaggagggagaaggagagggggaggaagaggaaggagaagggaagggcgaggaggaaggcgaagagggagagggggaaggcgaggaagaggaaggcgagggcgaaggagaggacggcgagggcgagggagaagaggaggaaggggaatgggaaggcgaagaagaggaaggcgaaggcgaaggcgaagaagagggcgaaggggagggcgaggagggcgaaggcgaaggggaggaagaggaaggcgaaggagaaggcgaggaagaagagggagaggaggaaggcgaggaggaaggagagggggaggaggagggagaaggcgagggcgaagaagaagaagagggagaagtggagggcgaagtcgagggggaggagggagaaggggaaggggaggaagaagagggcgaagaagaaggcgaggaaagagaaaaagagggagaaggcgaggaaaaccggagaaatagggaagaggaggaagaggaagagggaaagtaccaggagacaggcgaagaggaaaacgagcggcaggatggcgaggaatataagaaagtgagcaagatcaaaggatccgtcaagtacggcaagcacaaaacctatcagaagaaaagcgtgaccaacacacaggggaatggaaaagagcagaggagtaagatgcctgtgcagtcaaaacggctgctgaagaatggcccatctggaagtaaaaaattctggaacaatgtgctgccccactatctggaactgaaataa

SEQ ID NO: 4 - DNA, 934 bp, Artificial Sequence
  promoter sequence
attgacgtcaataatgacgtatgttcccatagtaacgccaatagggactttccattgacgtcaatgggtggagtatttacggtaaactgcccacttggcagtacatcaagtgtatcatatgccaagtacgccccctattgacgtcaatgacggtaaatggcccgcctggcattatgcccagtacatgaccttatgggactttcctacttggcagtacatctacgtattagtcatcgctattaccatggtcgaggtgagccccacgttctgcttcactctccccatctcccccccctccccacccccaattttgtatttatttattttttaattattttgtgcagcgatgggggcggggggggggggggggcgcgcgccaggcggggcggggcggggcgaggggcggggcggggcgaggcggagaggtgcggcggcagccaatcagagcggcgcgctccgaaagtttccttttatggcgaggcggcggcggcggcggccctataaaaagcgaagcgcgcggcgggcgggagtcgctgcgcgctgccttcgccccgtgccccgctccgccgccgcctcgcgccgcccgccccggctctgactgaccgcgttactcccacaggtgagcgggcgggacggcccttctcctccgggctgtaattagcgcttggtttaatgacggcttgtttcttttctgtggctgcgtgaaagccttgaggggctccgggagggccctttgtgcggggggagcggctcggggctgtccgcggggggacggctgccttcgggggggacggggcagggcggggttcggcttctggcgtgtgaccggcggctctagagcctctgctaaccatgttcatgccttcttctttttcctacagctcctgggcaacgtgctggttattgtgctgtctcatcattttggcaaagaatt

SEQ ID NO: 5 - DNA, 270 bp, Artificial Sequence
  Bovine Growth Hormone poly-A signal sequence
tcgctgatcagcctcgactgtgccttctagttgccagccatctgttgtttgcccctcccccgtgccttccttgaccctggaaggtgccactcccactgtcctttcctaataaaatgaggaaattgcatcgcattgtctgagtaggtgtcattctattctggggggtggggtggggcaggacagcaagggggaggattgggaagacaatagcaggcatgctggggatgcggtgggctctatggcttctgaggcggaaagaaccagctgggg

SEQ ID NO: 6 - DNA, 588 bp, Artificial Sequence
  woodchuck hepatitis postregulatory element (WPRE) example sequence
atcaacctctggattacaaaatttgtgaaagattgactggtattcttaactatgttgctccttttacgctatgtggatacgctgctttaatgcctttgtatcatgctattgcttcccgtatggctttcattttctcctccttgtataaatcctggttgctgtctctttatgaggagttgtggcccgttgtcaggcaacgtggcgtggtgtgcactgtgtttgctgacgcaacccccactggttggggcattgccaccacctgtcagctcctttccgggactttcgctttccccctccctattgccacggcggaactcatcgccgcctgccttgcccgctgctggacaggggctcggctgttgggcactgacaattccgtggtgttgtcggggaaatcatcgtcctttccttggctgctcgcctgtgttgccacctggattctgcgcgggacgtccttctgctacgtcccttcggccctcaatccagcggaccttccttcccgcggcctgctgccggctctgcggcctcttccgcgtcttcgccttcgccctcagacgagtcggatctccctttgggccgcctccccgc

SEQ ID NO: 7 - DNA, 199 bp, Artificial Sequence
  rhodopsin kinase (GRK1) promoter sequence
gggccccagaagcctggtggttgtttgtccttctcaggggaaaagtgaggcggccccttggaggaaggggccgggcagaatgatctaatcggattccaagcagctcaggggattgtctttttctagcaccttcttgccactcctaagcgtcctccgtgaccccggctgggatttagcctggtgctgtgtcagccccggg

SEQ ID NO: 8 - DNA, 235 bp, Artificial Sequence
  interphotoreceptor retinoid-binding protein (IRBP) promoter sequence
agcacagtgtctggcatgtagcaggaactaaaataatggcagtgattaatgttatgatatgcagacacaacacagcaagataagatgcaatgtaccttctgggtcaaaccaccctggccactcctccccgatacccagggttgatgtgcttgaattagacaggattaaaggcttactggagctggaagccttgccccaactcaggagtttagccccagaccttctgtccaccagc

SEQ ID NO: 9 - DNA, 3003 bp, Artificial Sequence
  a preferred RPGRORF15-encoding nucleotide sequence
atgagagagccagaggagctgatgccagacagtggagcagtgtttacattcggaaaatctaagttcgctgaaaataacccaggaaagttctggtttaaaaacgacgtgcccgtccacctgtcttgtggcgatgagcatagtgccgtggtcactgggaacaataagctgtacatgttcgggtccaacaactggggacagctggggctgggatccaaatctgctatctctaagccaacctgcgtgaaggcactgaaacccgagaaggtcaaactggccgcttgtggcagaaaccacactctggtgagcaccgagggcgggaatgtctatgccaccggaggcaacaatgagggacagctgggactgggggacactgaggaaaggaatacctttcacgtgatctccttctttacatctgagcataagatcaagcagctgagcgctggctccaacacatctgcagccctgactgaggacgggcgcctgttcatgtggggagataattcagagggccagattgggctgaaaaacgtgagcaatgtgtgcgtccctcagcaggtgaccatcggaaagccagtcagttggatttcatgtggctactatcatagcgccttcgtgaccacagatggcgagctgtacgtctttggggagcccgaaaacggaaaactgggcctgcctaaccagctgctgggcaatcaccggacaccccagctggtgtccgagatccctgaaaaagtgatccaggtcgcctgcgggggagagcatacagtggtcctgactgagaatgctgtgtataccttcggactgggccagtttggccagctggggctgggaaccttcctgtttgagacatccgaaccaaaagtgatcgagaacattcgcgaccagactatcagctacatttcctgcggagagaatcacaccgcactgatcacagacattggcctgatgtatacctttggcgatggacgacacgggaagctgggactgggactggagaacttcactaatcattttatccccaccctgtgttctaacttcctgcggttcatcgtgaaactggtcgcttgcggcgggtgtcacatggtggtcttcgctgcacctcataggggcgtggctaaggagatcgaatttgacgagattaacgatacatgcctgagcgtggcaactttcctgccatacagctccctgacttctggcaatgtgctgcagagaaccctgagtgcaaggatgcggagaagggagagggaacgctctcctgacagtttctcaatgcgacgaaccctgccacctatcgagggaacactgggactgagtgcctgcttcctgcctaactcagtgtttccacgatgtagcgagcggaatctgcaggagtctgtcctgagtgagcaggatctgatgcagccagaggaacccgactacctgctggatgagatgaccaaggaggccgaaatcgacaactctagtacagtggagtccctgggcgagactaccgatatcctgaatatgacacacattatgtcactgaacagcaatgagaagagtctgaaactgtcaccagtgcagaagcagaagaaacagcagactattggcgagctgactcaggacaccgccctgacagagaacgacgatagcgatgagtatgaggaaatgtccgagatgaaggaaggcaaagcttgtaagcagcatgtcagtcaggggatcttcatgacacagccagccacaactattgaggctttttcagacgaggaagtggagatccccgaggaaaaagagggcgcagaagattccaaggggaatggaattgaggaacaggaggtggaagccaacgaggaaaatgtgaaagtccacggaggcaggaaggagaaaacagaaatcctgtctgacgatctgactgacaaggccgaggtgtccgaaggcaaggcaaaatctgtcggagaggcagaagacggaccagagggacgaggggatggaacctgcgaggaaggctcaagcggggctgagcattggcaggacgaggaacgagagaagggcgaaaaggataaaggccgcggggagatggaacgacctggagagggcgaaaaagagctggcagagaaggaggaatggaagaaaagggacggcgaggaacaggagcagaaagaaagggagcagggccaccagaaggagcgcaaccaggagatggaagagggcggcgaggaagagcatggcgagggagaagaggaagagggcgatagagaagaggaagaggaaaaagaaggcgaagggaaggaggaaggagagggcgaggaagtggaaggcgagagggaaaaggaggaaggagaacggaagaaagaggaaagagccggcaaagaggaaaagggcgaggaagagggcgatcagggcgaaggcgaggaggaagagaccgagggccgcggggaagagaaagaggagggaggagaggtggagggcggagaggtcgaagagggaaagggcgagcgcgaagagggggaggaagaggaaggcgaaggagaaggcgaggaagaagagggagaggaggaaggcgaggaggaaggagagggggaggaggagggagaaggcgagggcgaagaagaagaagagggagaagtggagggcgaagtcgagggggaggagggagaaggggaaggggaggaagaagagggcgaagaagaaggcgaggaaagagaaaaagagggagaaggcgaggaaaaccggagaaatagggaagaggaggaagaggaagagggaaagtaccaggagacaggcgaagaggaaaacgagcggcaggatggcgaggaatataagaaagtgagcaagatcaaaggatccgtcaagtacggcaagcacaaaacctatcagaagaaaagcgtgaccaacacacaggggaatggaaaagagcagaggagtaagatgcctgtgcagtcaaaacggctgctgaagaatggcccatctggaagtaaaaaattctggaacaatgtgctgccccactatctggaactgaaataa

SEQ ID NO: 10 - DNA, 456 bp, Artificial Sequence
  deletion sequence
gaagaggaagagggcgagggcgaggaagaagagggcgagggggaagaagaggagggagagggcgaagaggaagagggggagggaaagggcgaagaggaaggagaggaaggggagggagaggaagagggggaggagggcgagggggaaggcgaggaggaagaaggagagggggaaggcgaagaggaaggcgagggggaaggagaggaggaagaaggggaaggcgaaggcgaagaggagggagaaggagagggggaggaagaggaaggagaagggaagggcgaggaggaaggcgaagagggagagggggaaggcgaggaagaggaaggcgagggcgaaggagaggacggcgagggcgagggagaagaggaggaaggggaatgggaaggcgaagaagaggaaggcgaaggcgaaggcgaagaagagggcgaaggggagggcgaggagggcgaaggcgaa

SEQ ID NO: 11 - DNA, 2517 bp, Artificial Sequence
  a preferred RPGRORF15-encoding nucleotide sequence
atgagagagccagaggagctgatgccagacagtggagcagtgtttacattcggaaaatctaagttcgctgaaaataacccaggaaagttctggtttaaaaacgacgtgcccgtccacctgtcttgtggcgatgagcatagtgccgtggtcactgggaacaataagctgtacatgttcgggtccaacaactggggacagctggggctgggatccaaatctgctatctctaagccaacctgcgtgaaggcactgaaacccgagaaggtcaaactggccgcttgtggcagaaaccacactctggtgagcaccgagggcgggaatgtctatgccaccggaggcaacaatgagggacagctgggactgggggacactgaggaaaggaatacctttcacgtgatctccttctttacatctgagcataagatcaagcagctgagcgctggctccaacacatctgcagccctgactgaggacgggcgcctgttcatgtggggagataattcagagggccagattgggctgaaaaacgtgagcaatgtgtgcgtccctcagcaggtgaccatcggaaagccagtcagttggatttcatgtggctactatcatagcgccttcgtgaccacagatggcgagctgtacgtctttggggagcccgaaaacggaaaactgggcctgcctaaccagctgctgggcaatcaccggacaccccagctggtgtccgagatccctgaaaaagtgatccaggtcgcctgcgggggagagcatacagtggtcctgactgagaatgctgtgtataccttcggactgggccagtttggccagctggggctgggaaccttcctgtttgagacatccgaaccaaaagtgatcgagaacattcgcgaccagactatcagctacatttcctgcggagagaatcacaccgcactgatcacagacattggcctgatgtatacctttggcgatggacgacacgggaagctgggactgggactggagaacttcactaatcattttatccccaccctgtgttctaacttcctgcggttcatcgtgaaactggtcgcttgcggcgggtgtcacatggtggtcttcgctgcacctcataggggcgtggctaaggagatcgaatttgacgagattaacgatacatgcctgagcgtggcaactttcctgccatacagctccctgacttctggcaatgtgctgcagagaaccctgagtgcaaggatgcggagaagggagagggaacgctctcctgacagtttctcaatgcgacgaaccctgccacctatcgagggaacactgggactgagtgcctgcttcctgcctaactcagtgtttccacgatgtagcgagcggaatctgcaggagtctgtcctgagtgagcaggatctgatgcagccagaggaacccgactacctgctggatgagatgaccaaggaggccgaaatcgacaactctagtacagtggagtccctgggcgagactaccgatatcctgaatatgacacacattatgtcactgaacagcaatgagaagagtctgaaactgtcaccagtgcagaagcagaagaaacagcagactattggcgagctgactcaggacaccgccctgacagagaacgacgatagcgatgagtatgaggaaatgtccgagatgaaggaaggcaaagcttgtaagcagcatgtcagtcaggggatcttcatgacacagccagccacaactattgaggctttttcagacgaggaagtggagatccccgaggaaaaagagggcgcagaagattccaaggggaatggaattgaggaacaggaggtggaagccaacgaggaaaatgtgaaagtccacggaggcaggaaggagaaaacagaaatcctgtctgacgatctgactgacaaggccgaggtgtccgaaggcaaggcaaaatctgtcggagaggcagaagacggaccagagggacgaggggatggaacctgcgaggaaggctcaagcggggctgagcattggcaggacgaggaacgagagaagggcgaaaaggataaaggccgcggggagatggaacgacctggagagggcgaaaaagaggaaggcgagggcgaagaagaagaagagggagaagtggagggcgaagtcgagggggaggagggagaaggggaaggggaggaagaagagggcgaagaagaaggcgaggaaagagaaaaagagggagaaggcgaggaaaaccggagaaatagggaagaggaggaagaggaagagggaaagtaccaggagacaggcgaagaggaaaacgagcggcaggatggcgaggaatataagaaagtgagcaagatcaaaggatccgtcaagtacggcaagcacaaaacctatcagaagaaaagcgtgaccaacacacaggggaatggaaaagagcagaggagtaagatgcctgtgcagtcaaaacggctgctgaagaatggcccatctggaagtaaaaaattctggaacaatgtgctgccccactatctggaactgaaataa

SEQ ID NO: 12 - DNA, 942 bp, Artificial Sequence
  deletion sequence
ctggcagagaaggaggaatggaagaaaagggacggcgaggaacaggagcagaaagaaagggagcagggccaccagaaggagcgcaaccaggagatggaagagggcggcgaggaagagcatggcgagggagaagaggaagagggcgatagagaagaggaagaggaaaaagaaggcgaagggaaggaggaaggagagggcgaggaagtggaaggcgagagggaaaaggaggaaggagaacggaagaaagaggaaagagccggcaaagaggaaaagggcgaggaagagggcgatcagggcgaaggcgaggaggaagagaccgagggccgcggggaagagaaagaggagggaggagaggtggagggcggagaggtcgaagagggaaagggcgagcgcgaagaggaagaggaagagggcgagggcgaggaagaagagggcgagggggaagaagaggagggagagggcgaagaggaagagggggagggaaagggcgaagaggaaggagaggaaggggagggagaggaagagggggaggagggcgagggggaaggcgaggaggaagaaggagagggggaaggcgaagaggaaggcgagggggaaggagaggaggaagaaggggaaggcgaaggcgaagaggagggagaaggagagggggaggaagaggaaggagaagggaagggcgaggaggaaggcgaagagggagagggggaaggcgaggaagaggaaggcgagggcgaaggagaggacggcgagggcgagggagaagaggaggaaggggaatgggaaggcgaagaagaggaaggcgaaggcgaaggcgaagaagagggcgaaggggagggcgaggagggcgaaggcgaaggggaggaagaggaaggcgaaggagaaggcgaggaagaagagggagaggaggaaggcgaggaggaaggagagggggaggaggaggga

SEQ ID NO: 13 - DNA, 3081 bp, Artificial Sequence
  a preferred RPGRORF15-encoding nucleotide sequence
atgagagagccagaggagctgatgccagacagtggagcagtgtttacattcggaaaatctaagttcgctgaaaataacccaggaaagttctggtttaaaaacgacgtgcccgtccacctgtcttgtggcgatgagcatagtgccgtggtcactgggaacaataagctgtacatgttcgggtccaacaactggggacagctggggctgggatccaaatctgctatctctaagccaacctgcgtgaaggcactgaaacccgagaaggtcaaactggccgcttgtggcagaaaccacactctggtgagcaccgagggcgggaatgtctatgccaccggaggcaacaatgagggacagctgggactgggggacactgaggaaaggaatacctttcacgtgatctccttctttacatctgagcataagatcaagcagctgagcgctggctccaacacatctgcagccctgactgaggacgggcgcctgttcatgtggggagataattcagagggccagattgggctgaaaaacgtgagcaatgtgtgcgtccctcagcaggtgaccatcggaaagccagtcagttggatttcatgtggctactatcatagcgccttcgtgaccacagatggcgagctgtacgtctttggggagcccgaaaacggaaaactgggcctgcctaaccagctgctgggcaatcaccggacaccccagctggtgtccgagatccctgaaaaagtgatccaggtcgcctgcgggggagagcatacagtggtcctgactgagaatgctgtgtataccttcggactgggccagtttggccagctggggctgggaaccttcctgtttgagacatccgaaccaaaagtgatcgagaacattcgcgaccagactatcagctacatttcctgcggagagaatcacaccgcactgatcacagacattggcctgatgtatacctttggcgatggacgacacgggaagctgggactgggactggagaacttcactaatcattttatccccaccctgtgttctaacttcctgcggttcatcgtgaaactggtcgcttgcggcgggtgtcacatggtggtcttcgctgcacctcataggggcgtggctaaggagatcgaatttgacgagattaacgatacatgcctgagcgtggcaactttcctgccatacagctccctgacttctggcaatgtgctgcagagaaccctgagtgcaaggatgcggagaagggagagggaacgctctcctgacagtttctcaatgcgacgaaccctgccacctatcgagggaacactgggactgagtgcctgcttcctgcctaactcagtgtttccacgatgtagcgagcggaatctgcaggagtctgtcctgagtgagcaggatctgatgcagccagaggaacccgactacctgctggatgagatgaccaaggaggccgaaatcgacaactctagtacagtggagtccctgggcgagactaccgatatcctgaatatgacacacattatgtcactgaacagcaatgagaagagtctgaaactgtcaccagtgcagaagcagaagaaacagcagactattggcgagctgactcaggacaccgccctgacagagaacgacgatagcgatgagtatgaggaaatgtccgagatgaaggaaggcaaagcttgtaagcagcatgtcagtcaggggatcttcatgacacagccagccacaactattgaggctttttcagacgaggaagtggagatccccgaggaaaaagagggcgcagaagattccaaggggaatggaattgaggaacaggaggtggaagccaacgaggaaaatgtgaaagtccacggaggcaggaaggagaaaacagaaatcctgtctgacgatctgactgacaaggccgaggtgtccgaaggcaaggcaaaatctgtcggagaggcagaagacggaccagagggacgaggggatggaacctgcgaggaaggctcaagcggggctgagcattggcaggacgaggaacgagagaagggcgaaaaggataaaggccgcggggagatggaacgacctggagagggcgaaaaagagctggcagagaaggaggaatggaagaaaagggacggcgaggaacaggagcagaaagaaagggagcagggccaccagaaggagcgcaaccaggagatggaagagggcggcgaggaagagcatggcgagggagaagaggaagagggcgatagagaagaggaagaggaaaaagaaggcgaagggaaggaggaaggagagggcgaggaagtggaaggcgagagggaaaaggaggaaggagaacggaagaaagaggaaagagccggcaaagaggaaaagggcgaggaagagggcgatcagggcgaaggcgaggaggaagagaccgagggccgcggggaagagaaagaggagggaggagaggtggagggcggagaggtcgaagagggaaagggcgagcgcgaagaggaagaggaagagggcgagggcgaggaagaagagggcgagggggaagaagaggagggagagggcgaagaggaagagggggagggaaagggcgaagaggaaggagaaggcgaggaagaagagggagaggaggaaggcgaggaggaaggagagggggaggaggagggagaaggcgagggcgaagaagaagaagagggagaagtggagggcgaagtcgagggggaggagggagaaggggaaggggaggaagaagagggcgaagaagaaggcgaggaaagagaaaaagagggagaaggcgaggaaaaccggagaaatagggaagaggaggaagaggaagagggaaagtaccaggagacaggcgaagaggaaaacgagcggcaggatggcgaggaatataagaaagtgagcaagatcaaaggatccgtcaagtacggcaagcacaaaacctatcagaagaaaagcgtgaccaacacacaggggaatggaaaagagcagaggagtaagatgcctgtgcagtcaaaacggctgctgaagaatggcccatctggaagtaaaaaattctggaacaatgtgctgccccactatctggaactgaaataa

SEQ ID NO: 14 - DNA, 378 bp, Artificial Sequence
  deletion sequence
ggagaggaaggggagggagaggaagagggggaggagggcgagggggaaggcgaggaggaagaaggagagggggaaggcgaagaggaaggcgagggggaaggagaggaggaagaaggggaaggcgaaggcgaagaggagggagaaggagagggggaggaagaggaaggagaagggaagggcgaggaggaaggcgaagagggagagggggaaggcgaggaagaggaaggcgagggcgaaggagaggacggcgagggcgagggagaagaggaggaaggggaatgggaaggcgaagaagaggaaggcgaaggcgaaggcgaagaagagggcgaaggggagggcgaggagggcgaaggcgaaggggaggaagaggaaggcgaa